European Patent Specification EP 3 430 043 B1, published August 30, 2023. Title: Anti-TNF-alpha antibodies and functional fragments thereof. Applicant: Tillotts Pharma AG. The sequence listing filed with the application follows.

SEQUENCE LISTING (62 sequences)

SEQ ID NO: 1 - protein, 11 aa, Artificial Sequence
  CDR
  MISC_FEATURE (7)..(7): Xaa is Phe, Ser, Gly or Tyr
  MISC_FEATURE (8)..(8): Xaa is Ser, Asn, Thr or Arg
  MISC_FEATURE (9)..(9): Xaa is Gly, Tyr, Ala, Asn or Ser
QASQSIXXXLA

SEQ ID NO: 2 - protein, 7 aa, Artificial Sequence
  CDR
  MISC_FEATURE (1)..(1): Xaa is Gly, Arg or Gln
  MISC_FEATURE (4)..(4): Xaa is Lys or Thr
  MISC_FEATURE (6)..(6): Xaa is Ala or Glu
XASXLXS

SEQ ID NO: 3 - protein, 15 aa, Artificial Sequence
  CDR
  MISC_FEATURE (6)..(6): Xaa is Ser or Thr
  MISC_FEATURE (8)..(8): Xaa is Ser or Ile
  MISC_FEATURE (9)..(9): Xaa is Ser, Thr or Asn
  MISC_FEATURE (13)..(13): Xaa is Ser or Phe
  MISC_FEATURE (14)..(14): Xaa is Tyr, Phe, Leu or Val
QSYYYXSXXSDGXXA

SEQ ID NO: 4 - protein, 10 aa, Artificial Sequence
  CDR
  MISC_FEATURE (5)..(5): Xaa is Asn or Ser
  MISC_FEATURE (6)..(6): Xaa is Asn or Thr
  MISC_FEATURE (10)..(10): Xaa is Gly, Cys or Ser
GIDFXXYGIX

SEQ ID NO: 5 - protein, 17 aa, Artificial Sequence
  CDR
  MISC_FEATURE (7)..(7): Xaa is Ala or Gly
  MISC_FEATURE (9)..(9): Xaa is Thr or Arg
  MISC_FEATURE (11)..(11): Xaa is Phe or Tyr
  MISC_FEATURE (13)..(13): Xaa is Asn or His
  MISC_FEATURE (15)..(15): Xaa is Val or Leu
YIYPGFXIXNXAXSXKG

SEQ ID NO: 6 - protein, 13 aa, Artificial Sequence
  CDR
  MISC_FEATURE (3)..(3): Xaa is Val, Ile or Leu
  MISC_FEATURE (5)..(5): Xaa is Ala or Ser
  MISC_FEATURE (6)..(6): Xaa is Thr or Ser
  MISC_FEATURE (7)..(7): Xaa is Asp or Ser
  MISC_FEATURE (8)..(8): Xaa is Trp or Ser
  MISC_FEATURE (9)..(9): Xaa is Gly or Ala
  MISC_FEATURE (11)..(11): Xaa is Phe, Leu or Tyr
  MISC_FEATURE (12)..(12): Xaa is Asp or Asn
DPXYXXXXXYXXL

SEQ ID NO: 7 - protein, 11 aa, Artificial Sequence
  CDR
QASQSIFSGLA

SEQ ID NO: 8 - protein, 7 aa, Artificial Sequence
  CDR
GASKLAS

SEQ ID NO: 9 - protein, 15 aa, Artificial Sequence
  CDR
QSYYYSSSSSDGSYA

SEQ ID NO: 10 - protein, 10 aa, Artificial Sequence
  CDR
GIDFNNYGIG

SEQ ID NO: 11 - protein, 17 aa, Artificial Sequence
  CDR
YIYPGFAITNFANSVKG

SEQ ID NO: 12 - protein, 13 aa, Artificial Sequence
  CDR
DPVYATSSGYFDL

SEQ ID NO: 13 - protein, 122 aa, Artificial Sequence
  humanized VH domain of clone 16-22-H05-sc02 and clone 16-22-H05-sc04
EVQLVESGGGLVQPGGSLRLSCKASGIDFNNYGIGWVRQAPGKGLEWITYIYPGFAITNFANSVKGRFTISSDNSKNTVYLQMNSLRAEDTAVYYCARDPVYATSSGYFDLWGQGTLVTVSS

SEQ ID NO: 14 - protein, 114 aa, Artificial Sequence
  humanized VL domain of clone 16-22-H05-sc02
DIQMTQSPSSLSASVGDRVTIKCQASQSIFSGLAWYQQKPGKAPKLLIYGASKLASGVPSRFSGSGSGTEFTLTISGLQPADFATYYCQSYYYSSSSSDGSYAFGGGTKLTVLG

SEQ ID NO: 15 - protein, 257 aa, Artificial Sequence
  humanized scFv of clone 16-22-H05-sc02
MDIQMTQSPSSLSASVGDRVTIKCQASQSIFSGLAWYQQKPGKAPKLLIYGASKLASGVPSRFSGSGSGTEFTLTISGLQPADFATYYCQSYYYSSSSSDGSYAFGGGTKLTVLGGGGGSGGGGSGGGGSGGGGSEVQLVESGGGLVQPGGSLRLSCKASGIDFNNYGIGWVRQAPGKGLEWITYIYPGFAITNFANSVKGRFTISSDNSKNTVYLQMNSLRAEDTAVYYCARDPVYATSSGYFDLWGQGTLVTVSS

SEQ ID NO: 16 - protein, 11 aa, Artificial Sequence
  CDR
QASQSISNYLA

SEQ ID NO: 17 - protein, 11 aa, Artificial Sequence
  CDR
QASQSISTALA

SEQ ID NO: 18 - protein, 11 aa, Artificial Sequence
  CDR
QASQSIGRNLA

SEQ ID NO: 19 - protein, 11 aa, Artificial Sequence
  CDR
QASQSISNSLA

SEQ ID NO: 20 - protein, 11 aa, Artificial Sequence
  CDR
QASQSIYSGLA

SEQ ID NO: 21 - protein, 11 aa, Artificial Sequence
  CDR
QASQSIGSNLA

SEQ ID NO: 22 - protein, 11 aa, Artificial Sequence
  CDR
QASQSISSSLA

SEQ ID NO: 23 - protein, 7 aa, Artificial Sequence
  CDR
RASTLAS

SEQ ID NO: 24 - protein, 7 aa, Artificial Sequence
  CDR
RASTLES

SEQ ID NO: 25 - protein, 7 aa, Artificial Sequence
  CDR
QASKLAS

SEQ ID NO: 26 - protein, 7 aa, Artificial Sequence
  CDR
RASKLAS

SEQ ID NO: 27 - protein, 15 aa, Artificial Sequence
  CDR
QSYYYSSSSSDGFFA

SEQ ID NO: 28 - protein, 15 aa, Artificial Sequence
  CDR
QSYYYSSSSSDGSFA

SEQ ID NO: 29 - protein, 15 aa, Artificial Sequence
  CDR
QSYYYSSSNSDGSLA

SEQ ID NO: 30 - protein, 15 aa, Artificial Sequence
  CDR
QSYYYSSISSDGSYA

SEQ ID NO: 31 - protein, 15 aa, Artificial Sequence
  CDR
QSYYYSSSSSDGSVA

SEQ ID NO: 32 - protein, 15 aa, Artificial Sequence
  CDR
QSYYYTSSTSDGSYA

SEQ ID NO: 33 - protein, 10 aa, Artificial Sequence
  CDR
GIDFSNYGIC

SEQ ID NO: 34 - protein, 10 aa, Artificial Sequence
  CDR
GIDFSNYGIS

SEQ ID NO: 35 - protein, 10 aa, Artificial Sequence
  CDR
GIDFSTYGIS

SEQ ID NO: 36 - protein, 10 aa, Artificial Sequence
  CDR
GIDFSNYGIG

SEQ ID NO: 37 - protein, 17 aa, Artificial Sequence
  CDR
YIYPGFGITNYANSVKG

SEQ ID NO: 38 - protein, 17 aa, Artificial Sequence
  CDR
YIYPGFGIRNYAHSVKG

SEQ ID NO: 39 - protein, 17 aa, Artificial Sequence
  CDR
YIYPGFGIRNYANSLKG

SEQ ID NO: 40 - protein, 17 aa, Artificial Sequence
  CDR
YIYPGFAIRNYANSVKG

SEQ ID NO: 41 - protein, 17 aa, Artificial Sequence
  CDR
YIYPGFGITNFANSVKG

SEQ ID NO: 42 - protein, 13 aa, Artificial Sequence
  CDR
DPIYASSSGYLDL

SEQ ID NO: 43 - protein, 13 aa, Artificial Sequence
  CDR
DPVYSSDWGYFNL

SEQ ID NO: 44 - protein, 13 aa, Artificial Sequence
  CDR
DPVYASSSGYLDL

SEQ ID NO: 45 - protein, 13 aa, Artificial Sequence
  CDR
DPLYATSSGYFDL

SEQ ID NO: 46 - protein, 13 aa, Artificial Sequence
  CDR
DPVYASSSGYFDL

SEQ ID NO: 47 - protein, 13 aa, Artificial Sequence
  CDR
DPVYASSSAYYNL

SEQ ID NO: 48 - protein, 13 aa, Artificial Sequence
  CDR
DPLYSTSSGYFNL

SEQ ID NO: 49 - protein, 20 aa, Artificial Sequence
  linker sequence in scFv
GGGGSGGGGSGGGGSGGGGS

SEQ ID NO: 50 - protein, 5 aa, Artificial Sequence
  linker sequence in diabody
GGGGS

SEQ ID NO: 51 - protein, 503 aa, Artificial Sequence
  Humanized diabody of clone 16-22-H05
MDIQMTQSPSSLSASVGDRVTIKCQASQSIFSGLAWYQQKPGKAPKLLIYGASKLASGVPSRFSGSGSGTEFTLTISGLQPADFATYYCQSYYYSSSSSDGSYAFGGGTKLTVLGGGGGSEVQLVESGGGLVQPGGSLRLSCKASGIDFNNYGIGWVRQAPGKGLEWITYIYPGFAITNFANSVKGRFTISSDNSKNTVYLQMNSLRAEDTAVYYCARDPVYATSSGYFDLWGQGTLVTVSSGGGGSGGGGSGGGGSGGGGSDIQMTQSPSSLSASVGDRVTIKCQASQSIFSGLAWYQQKPGKAPKLLIYGASKLASGVPSRFSGSGSGTEFTLTISGLQPADFATYYCQSYYYSSSSSDGSYAFGGGTKLTVLGGGGGSEVQLVESGGGLVQPGGSLRLSCKASGIDFNNYGIGWVRQAPGKGLEWITYIYPGFAITNFANSVKGRFTISSDNSKNTVYLQMNSLRAEDTAVYYCARDPVYATSSGYFDLWGQGTLVTVSS

SEQ ID NO: 52 - protein, 221 aa, Artificial Sequence
  light chain of humanized IgG of clone 16-22-H05
DIQMTQSPSSLSASVGDRVTIKCQASQSIFSGLAWYQQKPGKAPKLLIYGASKLASGVPSRFSGSGSGTEFTLTISGLQPADFATYYCQSYYYSSSSSDGSYAFGGGTKLTVLGRTVAAPSVFIFPPSDEQLKSGTASVVCLLNNFYPREAKVQWKVDNALQSGNSQESVTEQDSKDSTYSLSSTLTLSKADYEKHKVYACEVTHQGLSSPVTKSFNRGEC

SEQ ID NO: 53 - protein, 452 aa, Artificial Sequence
  heavy chain of humanized IgG of clone 16-22-H05
EVQLVESGGGLVQPGGSLRLSCKASGIDFNNYGIGWVRQAPGKGLEWITYIYPGFAITNFANSVKGRFTISSDNSKNTVYLQMNSLRAEDTAVYYCARDPVYATSSGYFDLWGQGTLVTVSSASTKGPSVFPLAPSSKSTSGGTAALGCLVKDYFPEPVTVSWNSGALTSGVHTFPAVLQSSGLYSLSSVVTVPSSSLGTQTYICNVNHKPSNTKVDKKVEPKSCDKTHTCPPCPAPELLGGPSVFLFPPKPKDQLMISRTPEVTCVVVDVSHEDPEVKFNWYVDGVEVHNAKTKPREEQYNSTYRVVSVLTVLHQDWLNGKEYKCKVSNKALPAPIEKTISKAKGQPREPQVYTLPPSREEMTKNQVSLTCLVKGFYPSDIAVEWESNGQPENNYKTTPPVLDSDGSFFLYSKLTVDKSRWQQGNVFSCSVLHEALHNHYTQKSLSLSPGK

SEQ ID NO: 54 - protein, 114 aa, Artificial Sequence
  humanized VL of clone 16-22-H05-sc04
DIQMTQSPSSLSASVGDRVTITCQASQSIFSGLAWYQQKPGKAPKLLIYGASKLASGVPSRFSGSGSGTEFTLTISGLQPADFATYYCQSYYYSSSSSDGSYAFGGGTKLTVLG

SEQ ID NO: 55 - protein, 257 aa, Artificial Sequence
  humanized scFv of clone 16-22-H05-sc04
MDIQMTQSPSSLSASVGDRVTITCQASQSIFSGLAWYQQKPGKAPKLLIYGASKLASGVPSRFSGSGSGTEFTLTISGLQPADFATYYCQSYYYSSSSSDGSYAFGGGTKLTVLGGGGGSGGGGSGGGGSGGGGSEVQLVESGGGLVQPGGSLRLSCKASGIDFNNYGIGWVRQAPGKGLEWITYIYPGFAITNFANSVKGRFTISSDNSKNTVYLQMNSLRAEDTAVYYCARDPVYATSSGYFDLWGQGTLVTVSS

SEQ ID NO: 56 - protein, 23 aa, Artificial Sequence
  Vk1 consensus sequence of framework I (Kabat positions 1-23)
DIQMTQSPSSLSASVGDRVTITC

SEQ ID NO: 57 - protein, 15 aa, Artificial Sequence
  Vk1 consensus sequence of framework II (Kabat positions 35-49)
WYQQKPGKAPKLLIY

SEQ ID NO: 58 - protein, 32 aa, Artificial Sequence
  Vk1 consensus sequence of framework III (Kabat positions 57-88)
GVPSRFSGSGSGTDFTLTISSLQPEDFATYYC

SEQ ID NO: 59 - protein, 10 aa, Artificial Sequence
  V lamda germline-based sequence of framework IV
FGTGTKVTVL

SEQ ID NO: 60 - protein, 10 aa, Artificial Sequence
  V lamda germline-based sequence of framework IV
FGGGTKLTVL

SEQ ID NO: 61 - protein, 10 aa, Artificial Sequence
  V lamda germline-based sequence of framework IV
FGGGTQLIIL

SEQ ID NO: 62 - protein, 10 aa, Artificial Sequence
  V lamda germline-based sequence of framework IV
FGSGTKVTVL